European Patent Application EP 4 407 028 A1, published July 31, 2024. Title: Method for producing modified human induced pluripotent stem cells. Applicant: CiRA Foundation. The sequence listing filed with the application follows.

SEQUENCE LISTING (2 sequences)

SEQ ID NO: 1 - RNA, 96 nt, Artificial Sequence
  synthesized RNA
gcgcgauccgcagguucucuguuuuagagcuagaaauagcaaguuaaaauaaggcuaguccguuaucaacuugaaaaaguggcaccgagucggugc

SEQ ID NO: 2 - RNA, 96 nt, Artificial Sequence
  synthesized RNA
gcugaacuggucgcaguugaguuuuagagcuagaaauagcaaguuaaaauaaggcuaguccguuaucaacuugaaaaaguggcaccgagucggugc